European Patent Application EP 4 585 220 A1, published July 16, 2025. Title: 항암 바이러스의 신규 용도. Applicant: 신라젠(주). The sequence listing filed with the application follows.

SEQUENCE LISTING (43 sequences)

SEQ ID NO: 1 - protein, 352 aa, synthetic construct
MTVARPSVPAALPLLGELPRLLLLVLLCLPAVWGDCGLPPDVPNAQPALEGRTSFPEDTVITYKCEESFVKIPGEKDSVICLKGSQWSDIEEFCNRSCEVPTRLNSASLKQPYITQNYFPVGTVVEYECRPGYRREPSLSPKLTCLQNLKWSTAVEFCKKKSCPNPGEIRNGQIDVPGGILFGATISFSCNTGYKLFGSTSSFCLISGSSVQWSDPLPECREIYCPAPPQIDNGIIQGERDHYGYRQSVTYACNKGFTMIGEHSIYCTVNNDEGEWSGPPPECRGKSLTSKVPPTVQKPTTVNVPTTEVSPTSQKTTTKTTTPNAQATRSTPVSRTTKHFHETTPNKGSGTT

SEQ ID NO: 2 - DNA, 1056 bp, synthetic construct
  source 1..1056: mol_type = other DNA
atgaccgtcgcgcggccgagcgtgcccgcggcgctgcccctcctcggggagctgccccggctgctgctgctggtgctgttgtgcctgccggccgtgtggggtgactgtggccttcccccagatgtacctaatgcccagccagctttggaaggccgtacaagttttcccgaggatactgtaataacgtacaaatgtgaagaaagctttgtgaaaattcctggcgagaaggactcagtgatctgccttaagggcagtcaatggtcagatattgaagagttctgcaatcgtagctgcgaggtgccaacaaggctaaattctgcatccctcaaacagccttatatcactcagaattattttccagtcggtactgttgtggaatatgagtgccgtccaggttacagaagagaaccttctctatcaccaaaactaacttgccttcagaatttaaaatggtccacagcagtcgaattttgtaaaaagaaatcatgccctaatccgggagaaatacgaaatggtcagattgatgtaccaggtggcatattatttggtgcaaccatctccttctcatgtaacacagggtacaaattatttggctcgacttctagtttttgtcttatttcaggcagctctgtccagtggagtgacccgttgccagagtgcagagaaatttattgtccagcaccaccacaaattgacaatggaataattcaaggggaacgtgaccattatggatatagacagtctgtaacgtatgcatgtaataaaggattcaccatgattggagagcactctatttattgtactgtgaataatgatgaaggagagtggagtggcccaccacctgaatgcagaggaaaatctctaacttccaaggtcccaccaacagttcagaaacctaccacagtaaatgttccaactacagaagtctcaccaacttctcagaaaaccaccacaaaaaccaccacaccaaatgctcaagcaacacggagtacacctgtttccaggacaaccaagcattttcatgaaacaaccccaaataaaggaagtggaaccact

SEQ ID NO: 3 - protein, 144 aa, synthetic construct [sequence omitted]

SEQ ID NO: 4 - DNA, 435 bp, synthetic construct
  source 1..435: mol_type = other DNA
atgtggctgcagagcctgctgctcttgggcactgtggcctgcagcatctctgcacccgcccgctcgcccagccccagcacgcagccctgggagcatgtgaatgccatccaggaggcccggcgtctcctgaacctgagtagagacactgctgctgagatgaatgaaacagtagaagtcatctcagaaatgtttgacctccaggagccgacctgcctacagacccgcctggagctgtacaagcagggcctgcggggcagcctcaccaagctcaagggccccttgaccatgatggccagccactacaagcagcactgccctccaaccccggaaacttcctgtgcaacccagactatcacctttgaaagtttcaaagagaacctgaaggactttctgcttgtcatcccctttgactgctgggagccagtccaggagtga

SEQ ID NO: 5 - DNA, 40 bp, synthetic construct
  source 1..40: mol_type = other DNA
aaaaattgaaattttattttttttttttggaatataaata

SEQ ID NO: 6 - DNA, 32 bp, synthetic construct
  source 1..32: mol_type = other DNA
ttttttttttttttttttttggcatataaata

SEQ ID NO: 7 - DNA, 104 bp, synthetic construct
  source 1..104: mol_type = other DNA
ccgtgcaataaattagaatatattttctacttttacgagaaattaattattgtatttattatttatgggtgaaaaacttactataaaaagcgggtgggtttgga

SEQ ID NO: 8 - protein, 141 aa, synthetic construct
MWLQNLLFLGIVVYSLSAPTRSPITVTRPWKHVEAIKEALNLLDDMPVTLNEEVEVVSNEFSFKKLTCVQTRLKIFEQGLRGNFTKLKGALNMTASYYQTYCPPTPETDCETQVTTYADFIDSLKTFLTDIPFECKKPVQK

SEQ ID NO: 9 - DNA, 426 bp, synthetic construct
  source 1..426: mol_type = other DNA
atgtggctgcagaatttacttttcctgggcattgtggtctacagcctctcagcacccacccgctcacccatcactgtcacccggccttggaagcatgtagaggccatcaaagaagccctgaacctcctggatgacatgcctgtcacattgaatgaagaggtagaagtcgtctctaacgagttctccttcaagaagctaacatgtgtgcagacccgcctgaagatattcgagcagggtctacggggcaatttcaccaaactcaagggcgccttgaacatgacagccagctactaccagacatactgccccccaactccggaaacggactgtgaaacacaagttaccacctatgcggatttcatagacagccttaaaacctttctgactgatatcccctttgaatgcaaaaaaccagtccaaaaatga

SEQ ID NO: 10 - protein, 40 aa, synthetic construct
LFDINVIGLIVILFIMFMLIFNVKSKLLWFLTGTFVTAFI

SEQ ID NO: 11 - DNA, 120 bp, synthetic construct
  source 1..120: mol_type = other DNA
ttgtttgatattaatgttataggtttgattgtaattttgtttattatgtttatgctcatctttaacgttaaatctaagctgttatggttccttacaggaacattcgttaccgcatttatc

SEQ ID NO: 12 - protein, 29 aa, synthetic construct
FAIIAIVFVFILTAILFFMSRRYSREKQN

SEQ ID NO: 13 - DNA, 87 bp, synthetic construct
  source 1..87: mol_type = other DNA
ttcgcaattattgccatagtattcgtgtttatacttaccgctattctcttttttatgagtcgacgatattcgcgagaaaaacaaaac

SEQ ID NO: 14 - protein, 35 aa, synthetic construct
LGAAITLVVISVIFYFISIYSRPKIKTNDINVRRR

SEQ ID NO: 15 - DNA, 105 bp, synthetic construct
  source 1..105: mol_type = other DNA
ttgggcgcggccataacattggttgtaatatctgttattttctattttatatctatttattcgcgtactaaaattaaaacaaatgatataaatgttcgtagacga

SEQ ID NO: 16 - protein, 37 aa, synthetic construct
PWFLVGVAIILVIFTVAICSIRRNLALKYRYGTFLYV

SEQ ID NO: 17 - DNA, 111 bp, synthetic construct
  source 1..111: mol_type = other DNA
ccgtggtttctagtgggtgtagcaattattctagttatttttactgtagctatttgttctattagacgaaatctggctcttaaatacagatacggaacgtttttatacgtt

SEQ ID NO: 18 - protein, 21 aa, synthetic construct
LKLHLISLLSLLVIWILIVAI

SEQ ID NO: 19 - DNA, 63 bp, synthetic construct
  source 1..63: mol_type = other DNA
ctaaaattgcatttgatcagtttattatctctcttggtaatatggatactaattgtagctatt

SEQ ID NO: 20 - protein, 67 aa, synthetic construct
VQFYMIVIGVIILAALFMYYAKRMLFTSTNDKIKLILANKENVHWTTYMDTFFRTSPMVIATTDMQN

SEQ ID NO: 21 - DNA, 201 bp, synthetic construct
  source 1..201: mol_type = other DNA
gttcagttttatatgattgttatcggtgttataatattggcagcgttgtttatgtactatgccaagcgtatgttgttcacatccaccaatgataaaatcaaacttattttagccaataaggaaaacgtccattggactacttacatggacacattctttagaacttctccgatggttattgctaccacggatatgcaaaac

SEQ ID NO: 22 - protein, 21 aa, synthetic construct
FVVVRAIASMIMYLVLGIALL

SEQ ID NO: 23 - DNA, 63 bp, synthetic construct
  source 1..63: mol_type = other DNA
ttcgtcgttgttagagccattgcgagcatgataatgtatttagtattaggtatagcattgctg

SEQ ID NO: 24 - protein, 21 aa, synthetic construct
MIGILLLIGICVAVTVAILYA

SEQ ID NO: 25 - DNA, 63 bp, synthetic construct
  source 1..63: mol_type = other DNA
atgattggtattcttttgttgatcggtatttgcgtagcagttaccgtcgccatcctatatgcg

SEQ ID NO: 26 - protein, 21 aa, synthetic construct
MITLFLILCYFILIFNIIVPA

SEQ ID NO: 27 - DNA, 63 bp, synthetic construct
  source 1..63: mol_type = other DNA
atgataactttatttttaatcctatgttatttcattcttatttttaatattatagtacctgca

SEQ ID NO: 28 - protein, 21 aa, synthetic construct
MNSLSIFFIVVATAAVCLLFI

SEQ ID NO: 29 - DNA, 63 bp, synthetic construct
  source 1..63: mol_type = other DNA
atgaactctctatcaattttttttattgtggtagcgacggctgcggtgtgtttactttttatc

SEQ ID NO: 30 - protein, 17 aa, synthetic construct
AVWTIIFIVLSQAGLDG

SEQ ID NO: 31 - DNA, 51 bp, synthetic construct
  source 1..51: mol_type = other DNA
gccgtatggaccattatttttatagtactttcgcaagcgggtttagacggc

SEQ ID NO: 32 - protein, 21 aa, synthetic construct
MASLLYLILFLLFVCISYYFT

SEQ ID NO: 33 - DNA, 63 bp, synthetic construct
  source 1..63: mol_type = other DNA
atggcatctttattatatcttattttatttttgttattcgtatgtatttcttattattttaca

SEQ ID NO: 34 - protein, 21 aa, synthetic construct
TSTLIFFVIILAISALLLWFQ

SEQ ID NO: 35 - DNA, 63 bp, synthetic construct
  source 1..63: mol_type = other DNA
acatcaacacttatattctttgttattatattggcaattagtgcgctattactctggtttcag

SEQ ID NO: 36 - protein, 21 aa, synthetic construct
YWLIIIFFIVLILLLLIYLYL

SEQ ID NO: 37 - DNA, 63 bp, synthetic construct
  source 1..63: mol_type = other DNA
tattggttaattattattttttttatagttcttattctactactattgatatatttgtattta

SEQ ID NO: 38 - protein, 21 aa, synthetic construct
IIDIKWLPIGLLALAILILAF

SEQ ID NO: 39 - DNA, 63 bp, synthetic construct
  source 1..63: mol_type = other DNA
attatagatatcaaatggcttccgattggattactagcgttagctattttaatattagcattt

SEQ ID NO: 40 - protein, 21 aa, synthetic construct
IVLFEVFVVFILIYVFFRSEL

SEQ ID NO: 41 - DNA, 63 bp, synthetic construct
  source 1..63: mol_type = other DNA
atagttttatttgaagtattcgttgtattcattctaatatatgtattttttagatctgaatta

SEQ ID NO: 42 - protein, 21 aa, synthetic construct
LVVIMFFIAFAFCSWLSYSYL

SEQ ID NO: 43 - DNA, 63 bp, synthetic construct
  source 1..63: mol_type = other DNA
ctcgtcgtaattatgttttttatagcgtttgccttctgtagttggctatcatatagctatctg